European Patent Application EP 4 119 507 A1, published January 18, 2023. Title: 一种黄酮苷类物质及其糖基转移酶基因在调控植物对杂草抗性中的应用. Applicant: 中国科学院植物研究所. The sequence listing filed with the application follows.

SEQUENCE LISTING (4 sequences)

SEQ ID NO: 1 - protein, 490 aa, Artificial sequence
MAPAMASSAATVVLIPFCVSGHLTPMLEVGKRMLRSRCCGDDDDGRPAMSLTVLLAQLPESHRAPEIDEIIRREAAGASEHSGFDVRFHCLPAEELPDFRGGEDFISRFMQQHASHAREAIAGLESRVAAVVLDWFCTTLLDVTRDLGLPGYVFFTSAASMLSLLLRLPALDKEVAVDFEEMGGAVDLPGLPPVPAALLPTPVMKKGCNYEWLVYHGSRFMEAAGIIVNTVAELEPAVLEAIADGRCVPGRRVPAIYTVGPVLSFKTPPEKPHECVRWLDAQPRASVVFLCFGSMGSFAPPQVLEIAAGLERSGHRFLWVLRGRPPAGSPYPTDADADELLPEGFLERTKGRGMVWPTWAPQKDILAHAAVGGFVTHGGWNSTLESLWHGVPMAPWPLYAEQHLNAFELVRDMGVAVEMEVDRKRGNLVEAAELERAVRCLMDEGSEEGRMAREKAAAAKAACRNAVDGGGSSIAALRKLTQEMAHMSSI

SEQ ID NO: 2 - DNA, 1473 bp, Artificial sequence
atggctccagcgatggcgagctcagcagcgacggtggtgctgatcccgttctgcgtctccggccacctcacgcccatgctggaagtcggcaagcggatgctgcgcagccgctgctgcggcgacgacgacgacggccgccccgccatgtcgctcaccgtgctcctcgcgcagctgccggagtcccaccgcgcgcccgagatcgacgagatcatccgccgtgaagcggccggcgcgtcggagcactccggcttcgacgtccggttccactgcctccccgccgaggagctcccggacttccgcggcggcgaggacttcatctcccggttcatgcagcagcacgcgtcgcacgccagggaggccatcgccggcctcgagtcccgcgtcgccgccgtggtcttggactggttctgcaccacgctcctcgacgtcacccgcgacctcggcctccccgggtacgtgttcttcacgtccgccgcctccatgctctcgctcctgctgcggttgccggcgctggacaaggaggtggccgtggatttcgaggagatgggaggcgccgtcgacttaccggggttgccgcctgtgccggcggctctgttgccgacgcctgtgatgaagaagggttgcaactacgagtggctcgtgtaccacgggagccgcttcatggaggctgcggggatcatcgtcaacacggtggccgagctcgagccggccgtcctcgaggccatcgccgacggccggtgcgtgccgggacgccgcgtcccggccatctacacggtcggccccgtgctgtcgttcaagacgccgcccgagaagccgcacgagtgcgtgcggtggctcgacgcgcagccgcgagcgtcggtcgtgttcctctgcttcgggagcatgggcagcttcgcgccgccgcaggtgctcgagatagccgccggcctcgagcgcagcgggcaccgcttcctgtgggtgctgcgcggccgtccacccgccggctcgccgtacccgacggacgccgacgccgacgagctcctcccggaggggttcctggagaggaccaaggggaggggcatggtgtggccgacgtgggcgccgcagaaggacatcctcgcccacgccgccgtgggaggcttcgtgacgcacggcgggtggaactcgacgctggagagcctgtggcacggcgtgccgatggcgccgtggccgctgtacgcggagcagcacctgaacgcgttcgagctcgtgcgcgacatgggcgtcgccgtggagatggaggtggacaggaagcggggcaacttggtggaggcggcggagctggagcgcgcggtgcggtgcctgatggacgagggatcggaggaggggaggatggcgagggagaaggcggcggcggcgaaggcggcgtgccggaacgccgtggacggaggcgggtcgtcgatagcggcgttgcggaagctcacgcaagaaatggcccacatgtcatccatatag

SEQ ID NO: 3 - protein, 489 aa, Artificial sequence
MASAMASSAATVVLIPFCVSGHLTPMLEVGKRMLRSRCCGDDDDGRPAMSLTVLLAQLPESHRAPEIDEIIRREAAGASEHSGFDVRFHCLPAEELPDFRGGEDFMSRFMQQHASHAREAIAGLESRVAAVVLDWFCTTLLDVTRDLGLPGYVFFTSAASMLSLLLRLPALDKEVAVDFEEMGGAVDLPGLPPVPAALLPTPVMKKGCNYEWLVYHGSRFMEAAGIIVNTVAELEPAVLEAIADGRCVPGRRVPAIYTVGPVLSFKTPPEKPHECVRWLDAQPRASVVFLCFGSMGSFAPPQVLEIAAGLERSGHRFLWVLRGQPAAGMPYPTDAVVDELLPEGFLERTKEKGLVWSKWAPQKEILAHPAVGGFATHCGWNSTLESLWNGVPLLPWPLYAEQHLNAFELVRDMGVAVEMEVDRKRGNLVEAAELERAVRCLMDEGSEGRMAREKAAAAKAACRNAVDGGGSSIAALRKLTQEMAHMSSI

SEQ ID NO: 4 - DNA, 2237 bp, Artificial sequence
gttcatgtctgaggggtgatttctgtagatttagaccattaaatttaatagaatagctttggcgtacattatggttattttttatcgacgagtaggcctacttgttctgaataaacatgacgccatgtgcggcgtatttcttttttttttttcaaagcaacccgggaaatctggacagtcagcgggaaaaacaagggtagtcagcatccattgtgacgtggtccattgactgcattcatgttacccctcccctctggcacccgatgtgcacgccaaaatgacaagcctccgcagggtctgtttagtttccaaataaaaattttccacaatgtcacactagatgtttggttatatatatatatatatatatatatatatatatatatatatatatatatatgtgtgtgtgtgtgtaaaatattaaatatataaaaaaactaattatatatattacatgtaaattacgagataaatcttttaagctcaattactccataatttgataatttattaatgacggattaattagacttaataaattcttctcgcagttcttagacgtaatatgtaatttattttattattaatttatatttaatatatatttaatactttaaatatgtatctatatccgatgttacatttcaaaaattttcgtttgcgaactaaaaaggccctcagtcctcagcttcagtgcctcacgcttgcaacaatatcgtcctccctgtccgtgtactgtgaatctgccatctgtgacttcgtgagacatggcttcagcgatggcgagctcagcagcgacggtcgtgctgatcccgttctgcgtctccggccacctcacgcccatgctggaagtcggcaagcggatgctgcgcagccgctgctgcggcgacgacgacgacggccgccccgccatgtcgctcaccgtgctcctcgcgcagctgccggagtcccaccgcgcgcccgagatcgacgagatcatccgccgtgaagcggccggcgcgtcggagcactccggcttcgacgtccggttccactgcctccccgccgaggagctcccggacttccgcggcggcgaggacttcatgtcccggttcatgcagcagcacgcgtcgcacgccagggaggccatcgccggcctcgagtcccgcgtcgccgccgtggtcttggactggttctgcaccacgctcctcgacgtcacccgcgacctcggcctccccgggtacgtgttcttcacgtccgccgcctccatgctctcgctcctgctgcggttgccggcgctggacaaggaggtggccgtggatttcgaggagatgggaggcgccgtcgacttaccggggttgccgccggtgccggcggctctgttgccgacgcctgtgatgaagaagggttgcaactacgagtggctcgtgtaccacgggagccgcttcatggaggctgcggggatcatcgtcaacacggtggccgagctcgagccggccgtcctcgaggccatcgccgacggccggtgcgtgccgggacgccgcgtcccggccatctacacggtcggccccgtgctgtcgttcaagacgccgcccgagaagccgcacgagtgcgtgcggtggctcgacgcgcagccgcgagcgtcggtcgtgttcctctgcttcgggagcatgggcagcttcgcgccgccgcaggtgctcgagatagccgccggcctcgagcgcagcggccaccgcttcctgtgggtactgcgcggccagccagccgccggcatgccatacccgacggacgccgtcgtcgacgagctcctccccgaggggttcttggagaggaccaaggagaagggcctcgtgtggtccaagtgggcgccgcagaaggagatcctcgcccaccctgccgtcggcggcttcgcgacgcactgcgggtggaactcgacgctggagagcctgtggaacggcgtgccgctactgccgtggccgctgtacgcggagcagcacctgaacgcgttcgagctcgtgcgcgacatgggcgtcgccgtggagatggaggtggacaggaagcggggcaacttggtggaggcggcggagctggagcgcgcggtgcggtgcctgatggacgagggatcggaggggaggatggcgagggagaaggcggcggcggcgaaggcggcgtgccggaacgccgtggacggaggcgggtcgtcgatagcggcgttgcggaagctcacgcaagaaatggcccacatgtcatccatatag